European Patent Application EP 4 643 871 A1, published November 5, 2025. Title: A Composition Comprising Aflibercept and a Variant thereof, and Related Methods and Uses. Applicant: QILU PHARMACEUTICAL CO., LTD. The sequence listing filed with the application follows.

SEQUENCE LISTING (6 sequences)

SEQ ID NO: 1 - protein, 432 aa, synthetic construct
SDTGRPFVEMYSEIPEIIHMTEGRELVIPCRVTSPNITVTLKKFPLDTLIPDGKRIIWDSRKGFIISNATYKEIGLLTCEATVNGHLYKTNYLTHRQTNTIIDVVLSPSHGIELSVGEKLVLNCTARTELNVGIDFNWEYPSSKHQHKKLVNRDLKTQSGSEMKKFLSTLTIDGVTRSDQGLYTCAASSGLMTKKNSTFVRVHEKDKTHTCPPCPAPELLGGPSVFLFPPKPKDTLMISRTPEVTCVVVDVSHEDPEVKFNWYVDGVEVHNAKTKPREEQYNSTYRVVSVLTVLHQDWLNGKEYKCKVSNKALPAPIEKTISKAKGQPREPQVYTLPPSRDELTKNQVSLTCLVKGFYPSDIAVEWESNGQPENNYKTTPPVLDSDGSFFLYSKLTVDKSRWQQGNVFSCSVMHEALHNHYTQKSLSLSPGK

SEQ ID NO: 2 - protein, 333 aa, synthetic construct
TIIDVVLSPSHGIELSVGEKLVLNCTARTELNVGIDFNWEYPSSKHQHKKLVNRDLKTQSGSEMKKFLSTLTIDGVTRSDQGLYTCAASSGLMTKKNSTFVRVHEKDKTHTCPPCPAPELLGGPSVFLFPPKPKDTLMISRTPEVTCVVVDVSHEDPEVKFNWYVDGVEVHNAKTKPREEQYNSTYRVVSVLTVLHQDWLNGKEYKCKVSNKALPAPIEKTISKAKGQPREPQVYTLPPSRDELTKNQVSLTCLVKGFYPSDIAVEWESNGQPENNYKTTPPVLDSDGSFFLYSKLTVDKSRWQQGNVFSCSVMHEALHNHYTQKSLSLSPGK

SEQ ID NO: 3 - protein, 432 aa, synthetic construct
SDTGRPFVEMYSEIPEIIHMTEGRELVIPCRVTSPNITVTLKKFPLDTLIPDGKRIIWDSRKGFIISNATYKEIGLLTCEATVNGHLYKTNYLTHRQTNTIIDVVLSPSHGIELSVGEKLVLNCTARTELNVGIDFNWEYPSSKHQHKKLVNRDLKTQSGSEMKKFLSTLTIDGVTRSDQGLYTCAASSGLMTKKNSTFVRVHEKDKTHTCPPCPAPELLGGPSVFLFPPKPKDTLMISRTPEVTCVVVDVSHEDPEVKFNWYVDGVEVHNAKTKPREEQYNSTYRVVSVLTVLHQDWLNGKEYKCKVSNKALPAPIEKTISKAKGQPREPQVYTLPPCRDELTKNQVSLWCLVKGFYPSDIAVEWESNGQPENNYKTTPPVLDSDGSFFLYSKLTVDKSRWQQGNVFSCSVMHEALHNHYTQKSLSLSPGK

SEQ ID NO: 4 - protein, 333 aa, synthetic construct
TIIDVVLSPSHGIELSVGEKLVLNCTARTELNVGIDFNWEYPSSKHQHKKLVNRDLKTQSGSEMKKFLSTLTIDGVTRSDQGLYTCAASSGLMTKKNSTFVRVHEKDKTHTCPPCPAPELLGGPSVFLFPPKPKDTLMISRTPEVTCVVVDVSHEDPEVKFNWYVDGVEVHNAKTKPREEQYNSTYRVVSVLTVLHQDWLNGKEYKCKVSNKALPAPIEKTISKAKGQPREPQVCTLPPSRDELTKNQVSLSCAVKGFYPSDIAVEWESNGQPENNYKTTPPVLDSDGSFFLVSKLTVDKSRWQQGNVFSCSVMHEALHNRYTQKSLSLSPGK

SEQ ID NO: 5 - protein, 23 aa, synthetic construct
QTNTIIDVVLSPSHGIELSVGEK

SEQ ID NO: 6 - protein, 20 aa, synthetic construct
TIIDVVLSPSHGIELSVGEK